European Patent Application EP 4 309 741 A1, published January 24, 2024. Title: Cyclic compounds with selective KRAS inhibitory effects over HRAS and NRAS. Applicant: CHUGAI SEIYAKU KABUSHIKI KAISHA. The sequence listing filed with the application follows.

SEQUENCE LISTING (6 sequences)

SEQ ID NO: 1 - DNA, 615 bp, Artificial sequence
  HAT_Linker_Thrombin_Linker_hKRAS
atgaaagatcacctgattcacaatgtccataaagaagaacacgcccatgctcactcgtctggcagcctggtcccgcgtggttcgtcaggcgggagcaccgagtacaaactggtggttgtaggtgccggtggtgttggcaagagcgcgctgacgatccagttgattcaaaaccactttgtcgatgagtatgacccgacgatcgaggacagctaccgtaaacaagttgtgatcgatggcgagacttgcctgctggatattctggacacggctggccaagaagaatacagcgcgatgcgtgaccagtacatgcgcaccggtgagggtttcctgtgtgttttcgcaattaacaatacgaaatcctttgaggatattcatcactatcgtgaacagatcaagcgtgttaaagacagcgaagatgtcccgatggtgttggtgggcaataagtgcgatctgccgagccgcaccgtcgataccaaacaggcacaggacctggcgcgcagctatggtatcccgttcattgaaacctctgcgaaaacccgccaaggtgtcgacgacgccttttacaccctggtgcgtgagatccgtaagcataaggaaaagatgagcaaagacggc

SEQ ID NO: 2 - protein, 205 aa, Artificial sequence
  HAT_Linker_Thrombin_Linker_hKRAS
MKDHLIHNVHKEEHAHAHSSGSLVPRGSSGGSTEYKLVVVGAGGVGKSALTIQLIQNHFVDEYDPTIEDSYRKQVVIDGETCLLDILDTAGQEEYSAMRDQYMRTGEGFLCVFAINNTKSFEDIHHYREQIKRVKDSEDVPMVLVGNKCDLPSRTVDTKQAQDLARSYGIPFIETSAKTRQGVDDAFYTLVREIRKHKEKMSKDG

SEQ ID NO: 3 - protein, 179 aa, Artificial sequence
  Linker_hKRAS
GSSGGSTEYKLVVVGAGGVGKSALTIQLIQNHFVDEYDPTIEDSYRKQVVIDGETCLLDILDTAGQEEYSAMRDQYMRTGEGFLCVFAINNTKSFEDIHHYREQIKRVKDSEDVPMVLVGNKCDLPSRTVDTKQAQDLARSYGIPFIETSAKTRQGVDDAFYTLVREIRKHKEKMSKDG

SEQ ID NO: 4 - protein, 189 aa, Homo sapiens
MTEYKLVVVGAGGVGKSALTIQLIQNHFVDEYDPTIEDSYRKQVVIDGETCLLDILDTAGQEEYSAMRDQYMRTGEGFLCVFAINNSKSFADINLYREQIKRVKDSDDVPMVLVGNKCDLPTRTVDTKQAHELAKSYGIPFIETSAKTRQGVEDAFYTLVREIRQYRMKKLNSSDDGTQGCMGLPCVVM

SEQ ID NO: 5 - protein, 189 aa, Homo sapiens
MTEYKLVVVGAGGVGKSALTIQLIQNHFVDEYDPTIEDSYRKQVVIDGETCLLDILDTAGQEEYSAMRDQYMRTGEGFLCVFAINNTKSFEDIHQYREQIKRVKDSDDVPMVLVGNKCDLAARTVESRQAQDLARSYGIPYIETSAKTRQGVEDAFYTLVREIRQHKLRKLNPPDESGPGCMSCKCVLS

SEQ ID NO: 6 - protein, 189 aa, Homo sapiens [sequence omitted]